European Patent Specification EP 4 132 920 B1, published August 13, 2025. Title: INHIBITORS OF SARM1. Applicant: DISARM THERAPEUTICS, INC. The sequence listing filed with the application follows.

SEQUENCE LISTING (1 sequence)

SEQ ID NO: 1 - DNA, 13028 bp, Artificial Sequence
  Synthetic Construct
gcgatcgcggctcccgacatcttggaccattagctccacaggtatcttcttccctctagtggtcataacagcagcttcagctacctctcaattcaaaaaacccctcaagacccgtttagaggccccaaggggttatgctatcaatcgttgcgttacacacacaaaaaaccaacacacatccatcttcgatggatagcgattttattatctaactgctgatcgagtgtagccagatctagtaatcaattacggggtcattagttcatagcccatatatggagttccgcgttacataacttacggtaaatggcccgcctggctgaccgcccaacgacccccgcccattgacgtcaataatgacgtatgttcccatagtaacgccaatagggactttccattgacgtcaatgggtggagtatttacggtaaactgcccacttggcagtacatcaagtgtatcatatgccaagtacgccccctattgacgtcaatgacggtaaatggcccgcctggcattatgcccagtacatgaccttatgggactttcctacttggcagtacatctacgtattagtcatcgctattaccatgctgatgcggttttggcagtacatcaatgggcgtggatagcggtttgactcacggggatttccaagtctccaccccattgacgtcaatgggagtttgttttggcaccaaaatcaacgggactttccaaaatgtcgtaacaactccgccccattgacgcaaatgggcggtaggcgtgtacggtgggaggtctatataagcagagctggtttagtgaaccgtcagatcagatctttgtcgatcctaccatccactcgacacacccgccagcggccgctgccaagcttccgagctctcgaattcaaaggaggtacccaccatggccatgcatcaccaccaccatcatagctccggcgtcgacctcggcaccgagaatttatatttccaaagcggcctcaatgatatcttcgaggcccagaagatcgagtggcacgagggcagctccgacctcgccgtgcccggtcccgatggaggcggaggcactggtccttggtgggctgctggcggcagaggccctagagaagtgagccccggtgctggcaccgaggtgcaagacgctctggagagggctctgcccgaactgcagcaagctctgtccgctttaaagcaagctggaggagctagagccgtcggcgccggactggccgaagtgttccagctcgtggaggaagcttggttattacccgctgtgggaagagaggtcgcccaaggtctgtgtgacgccattcgtctggacggaggtttagacttattactgaggctgctgcaagctcccgaactggagacaagggtccaagctgctcgtctgctggagcagatcctcgtggccgagaatcgtgacagagtggctagaatcggtttaggcgtcatcctcaatttagccaaagagagggagcccgttgagctggccagaagcgtcgctggcatcctcgagcacatgttcaagcattccgaggagacttgtcagagactggtcgccgccggaggactcgatgctgttttatactggtgcagaaggacagaccccgctttactgaggcattgtgctctggccctcggcaattgcgctttacatggaggccaagccgtccagagaaggatggtggagaaaagagccgccgagtggctgttccctttagccttctccaaagaagacgaactgttacgtctgcatgcttgtctcgctgtcgctgttttagccaccaacaaggaggtggaaagggaagtggaaagaagcggaacactggctttagtcgaacctctggtggcttctttagatcccggaaggtttgccagatgtctggtcgacgccagcgatacctcccaaggaagaggccccgacgatctccagagactggtgcctctgctggacagcaatcgtctggaggcccaatgtattggcgccttctatctctgcgccgaagccgccatcaagtctttacaaggtaagaccaaggtgttctccgacattggagccatccaatctttaaagaggctggtgagctattccaccaacggcacaaaaagcgctttagccaaaagagctttaagactgctgggcgaagaggtgcctaggcccattttaccttccgtgcctagctggaaggaggccgaggtgcagacttggctgcagcagatcggctttagcaaatattgcgaatcctttagggagcagcaagttgacggcgatttattattaaggctgaccgaggaagagctccagacagatttaggcatgaaaagcggcatcactcgtaagaggttctttcgtgagctcaccgaactgaagaccttcgccaactactccacttgtgatcgtagcaatttagctgattggctcggatccctcgatcccagatttcgtcagtacacctatggactcgtctcttgtggactggacagatctttactgcatcgtgtgagcgagcaacagctgctggaagattgcggcatccatttaggagtgcacagagccagaattctgaccgccgctagagagatgctgcattcccctctcccttgtaccggaggcaagcctagcggagacacccccgacgtgttcatcagctatcgtagaaacagcggaagccagctggcctctttactgaaggtccatttacagctgcacggatttagcgtcttcatcgacgtggagaaactggaggctggcaagttcgaggacaagctgatccagtccgtgatgggcgctaggaatttcgttttagtgctcagccccggcgctctggataaatgcatgcaagatcatgactgtaaggactgggtccacaaggaaatcgtgaccgctctgtcttgtggcaagaacatcgtccccatcatcgacggcttcgaatggcccgagcctcaagttctccccgaagatatgcaagctgttttaaccttcaatggaatcaagtggagccacgagtaccaagaagccacaatcgagaagatcattcgttttctgcaaggtagatcctccagagattcctccgctggcagcgacacatctttagagggcgccgcccctatgggtcctacctaataatctagaagttgtctcctcctgcactgactgactgatacaatcgatttctggatccgcaggcctctgctagcttgactgactgagatacagcgtaccttcagctcacagacatgataagatacattgatgagtttggacaaaccacaactagaatgcagtgaaaaaaatgctttatttgtgaaatttgtgatgctattgctttatttgtaaccattataagctgcaataaacaagttaacaacaacaattgcattcattttatgtttcaggttcagggggaggtgtgggaggttttttaaagcaagtaaaacctctacaaatgtggtattggcccatctctatcggtatcgtagcataaccccttggggcctctaaacgggtcttgaggggttttttgtgcccctcgggccggattgctatctaccggcattggcgcagaaaaaaatgcctgatgcgacgctgcgcgtcttatactcccacatatgccagattcagcaacggatacggcttccccaacttgcccacttccatacgtgtcctccttaccagaaatttatccttaaggtcgtcagctatcctgcaggcgatctctcgatttcgatcaagacattcctttaatggtcttttctggacaccactaggggtcagaagtagttcatcaaactttcttccctccctaatctcattggttaccttgggctatcgaaacttaattaaccagtcaagtcagctacttggcgagatcgacttgtctgggtttcgactacgctcagaattgcgtcagtcaagttcgatctggtccttgctattgcacccgttctccgattacgagtttcatttaaatcatgtgagcaaaaggccagcaaaaggccaggaaccgtaaaaaggccgcgttgctggcgtttttccataggctccgcccccctgacgagcatcacaaaaatcgacgctcaagtcagaggtggcgaaacccgacaggactataaagataccaggcgtttccccctggaagctccctcgtgcgctctcctgttccgaccctgccgcttaccggatacctgtccgcctttctcccttcgggaagcgtggcgctttctcatagctcacgctgtaggtatctcagttcggtgtaggtcgttcgctccaagctgggctgtgtgcacgaaccccccgttcagcccgaccgctgcgccttatccggtaactatcgtcttgagtccaacccggtaagacacgacttatcgccactggcagcagccactggtaacaggattagcagagcgaggtatgtaggcggtgctacagagttcttgaagtggtggcctaactacggctacactagaagaacagtatttggtatctgcgctctgctgaagccagttaccttcggaaaaagagttggtagctcttgatccggcaaacaaaccaccgctggtagcggtggtttttttgtttgcaagcagcagattacgcgcagaaaaaaaggatctcaagaagatcctttgatcttttctacggggtctgacgctcagtggaacgaaaactcacgttaagggattttggtcatgagattatcaaaaaggatcttcacctagatccttttaaattaaaaatgaagttttaaatcaatctaaagtatatatgagtaaacttggtctgacagttaccaatgcttaatcagtgaggcacctatctcagcgatctgtctatttcgttcatccatagttgcatttaaatttccgaactctccaaggccctcgtcggaaaatcttcaaacctttcgtccgatccatcttgcaggctacctctcgaacgaactatcgcaagtctcttggccggccttgcgccttggctattgcttggcagcgcctatcgccaggtattactccaatcccgaatatccgagatcgggatcacccgagagaagttcaacctacatcctcaatcccgatctatccgagatccgaggaatatcgaaatcggggcgcgcctggtgtaccgagaacgatcctctcagtgcgagtctcgacgatccatatcgttgcttggcagtcagccagtcggaatccagcttgggacccaggaagtccaatcgtcagatattgtactcaagcctggtcacggcagcgtaccgatctgtttaaacctagatattgatagtctgatcggtcaacgtataatcgagtcctagcttttgcaaacatctatcaagagacaggatcagcaggaggctttcgcatgagtattcaacatttccgtgtcgcccttattcccttttttgcggcattttgccttcctgtttttgctcacccagaaacgctggtgaaagtaaaagatgctgaagatcagttgggtgcgcgagtgggttacatcgaactggatctcaacagcggtaagatccttgagagttttcgccccgaagaacgctttccaatgatgagcacttttaaagttctgctatgtggcgcggtattatcccgtattgacgccgggcaagagcaactcggtcgccgcatacactattctcagaatgacttggttgagtattcaccagtcacagaaaagcatcttacggatggcatgacagtaagagaattatgcagtgctgccataaccatgagtgataacactgcggccaacttacttctgacaacgattggaggaccgaaggagctaaccgcttttttgcacaacatgggggatcatgtaactcgccttgatcgttgggaaccggagctgaatgaagccataccaaacgacgagcgtgacaccacgatgcctgtagcaatggcaacaaccttgcgtaaactattaactggcgaactacttactctagcttcccggcaacagttgatagactggatggaggcggataaagttgcaggaccacttctgcgctcggcccttccggctggctggtttattgctgataaatctggagccggtgagcgtgggtctcgcggtatcattgcagcactggggccagatggtaagccctcccgtatcgtagttatctacacgacggggagtcaggcaactatggatgaacgaaatagacagatcgctgagataggtgcctcactgattaagcattggtaaccgattctaggtgcattggcgcagaaaaaaatgcctgatgcgacgctgcgcgtcttatactcccacatatgccagattcagcaacggatacggcttccccaacttgcccacttccatacgtgtcctccttaccagaaatttatccttaagatcccgaatcgtttaaactcgactctggctctatcgaatctccgtcgtttcgagcttacgcgaacagccgtggcgctcatttgctcgtcgggcatcgaatctcgtcagctatcgtcagcttacctttttggcagcgatcgcggctcccgacatcttggaccattagctccacaggtatcttcttccctctagtggtcataacagcagcttcagctacctctcaattcaaaaaacccctcaagacccgtttagaggccccaaggggttatgctatcaatcgttgcgttacacacacaaaaaaccaacacacatccatcttcgatggatagcgattttattatctaactgctgatcgagtgtagccagatctagtaatcaattacggggtcattagttcatagcccatatatggagttccgcgttacataacttacggtaaatggcccgcctggctgaccgcccaacgacccccgcccattgacgtcaataatgacgtatgttcccatagtaacgccaatagggactttccattgacgtcaatgggtggagtatttacggtaaactgcccacttggcagtacatcaagtgtatcatatgccaagtacgccccctattgacgtcaatgacggtaaatggcccgcctggcattatgcccagtacatgaccttatgggactttcctacttggcagtacatctacgtattagtcatcgctattaccatgctgatgcggttttggcagtacatcaatgggcgtggatagcggtttgactcacggggatttccaagtctccaccccattgacgtcaatgggagtttgttttggcaccaaaatcaacgggactttccaaaatgtcgtaacaactccgccccattgacgcaaatgggcggtaggcgtgtacggtgggaggtctatataagcagagctggtttagtgaaccgtcagatcagatctttgtcgatcctaccatccactcgacacacccgccagcggccgctgccaagcttccgagctctcgaattcaaaggaggtacccaccatggccatgcatcaccaccaccatcatagctccggcgtcgacctcggcaccgagaatttatatttccaaagcggcctcaatgatatcttcgaggcccagaagatcgagtggcacgagggcagctccgacctcgccgtgcccggtcccgatggaggcggaggcactggtccttggtgggctgctggcggcagaggccctagagaagtgagccccggtgctggcaccgaggtgcaagacgctctggagagggctctgcccgaactgcagcaagctctgtccgctttaaagcaagctggaggagctagagccgtcggcgccggactggccgaagtgttccagctcgtggaggaagcttggttattacccgctgtgggaagagaggtcgcccaaggtctgtgtgacgccattcgtctggacggaggtttagacttattactgaggctgctgcaagctcccgaactggagacaagggtccaagctgctcgtctgctggagcagatcctcgtggccgagaatcgtgacagagtggctagaatcggtttaggcgtcatcctcaatttagccaaagagagggagcccgttgagctggccagaagcgtcgctggcatcctcgagcacatgttcaagcattccgaggagacttgtcagagactggtcgccgccggaggactcgatgctgttttatactggtgcagaaggacagaccccgctttactgaggcattgtgctctggccctcggcaattgcgctttacatggaggccaagccgtccagagaaggatggtggagaaaagagccgccgagtggctgttccctttagccttctccaaagaagacgaactgttacgtctgcatgcttgtctcgctgtcgctgttttagccaccaacaaggaggtggaaagggaagtggaaagaagcggaacactggctttagtcgaacctctggtggcttctttagatcccggaaggtttgccagatgtctggtcgacgccagcgatacctcccaaggaagaggccccgacgatctccagagactggtgcctctgctggacagcaatcgtctggaggcccaatgtattggcgccttctatctctgcgccgaagccgccatcaagtctttacaaggtaagaccaaggtgttctccgacattggagccatccaatctttaaagaggctggtgagctattccaccaacggcacaaaaagcgctttagccaaaagagctttaagactgctgggcgaagaggtgcctaggcccattttaccttccgtgcctagctggaaggaggccgaggtgcagacttggctgcagcagatcggctttagcaaatattgcgaatcctttagggagcagcaagttgacggcgatttattattaaggctgaccgaggaagagctccagacagatttaggcatgaaaagcggcatcactcgtaagaggttctttcgtgagctcaccgaactgaagaccttcgccaactactccacttgtgatcgtagcaatttagctgattggctcggatccctcgatcccagatttcgtcagtacacctatggactcgtctcttgtggactggacagatctttactgcatcgtgtgagcgagcaacagctgctggaagattgcggcatccatttaggagtgcacagagccagaattctgaccgccgctagagagatgctgcattcccctctcccttgtaccggaggcaagcctagcggagacacccccgacgtgttcatcagctatcgtagaaacagcggaagccagctggcctctttactgaaggtccatttacagctgcacggatttagcgtcttcatcgacgtggagaaactggaggctggcaagttcgaggacaagctgatccagtccgtgatgggcgctaggaatttcgttttagtgctcagccccggcgctctggataaatgcatgcaagatcatgactgtaaggactgggtccacaaggaaatcgtgaccgctctgtcttgtggcaagaacatcgtccccatcatcgacggcttcgaatggcccgagcctcaagttctccccgaagatatgcaagctgttttaaccttcaatggaatcaagtggagccacgagtaccaagaagccacaatcgagaagatcattcgttttctgcaaggtagatcctccagagattcctccgctggcagcgacacatctttagagggcgccgcccctatgggtcctacctaataatctagaagttgtctcctcctgcactgactgactgatacaatcgatttctggatccgcaggcctctgctagcttgactgactgagatacagcgtaccttcagctcacagacatgataagatacattgatgagtttggacaaaccacaactagaatgcagtgaaaaaaatgctttatttgtgaaatttgtgatgctattgctttatttgtaaccattataagctgcaataaacaagttaacaacaacaattgcattcattttatgtttcaggttcagggggaggtgtgggaggttttttaaagcaagtaaaacctctacaaatgtggtattggcccatctctatcggtatcgtagcataaccccttggggcctctaaacgggtcttgaggggttttttgtgcccctcgggccggattgctatctaccggcattggcgcagaaaaaaatgcctgatgcgacgctgcgcgtcttatactcccacatatgccagattcagcaacggatacggcttccccaacttgcccacttccatacgtgtcctccttaccagaaatttatccttaaggtcgtcagctatcctgcaggcgatctctcgatttcgatcaagacattcctttaatggtcttttctggacaccactaggggtcagaagtagttcatcaaactttcttccctccctaatctcattggttaccttgggctatcgaaacttaattaaccagtcaagtcagctacttggcgagatcgacttgtctgggtttcgactacgctcagaattgcgtcagtcaagttcgatctggtccttgctattgcacccgttctccgattacgagtttcatttaaatcatgtgagcaaaaggccagcaaaaggccaggaaccgtaaaaaggccgcgttgctggcgtttttccataggctccgcccccctgacgagcatcacaaaaatcgacgctcaagtcagaggtggcgaaacccgacaggactataaagataccaggcgtttccccctggaagctccctcgtgcgctctcctgttccgaccctgccgcttaccggatacctgtccgcctttctcccttcgggaagcgtggcgctttctcatagctcacgctgtaggtatctcagttcggtgtaggtcgttcgctccaagctgggctgtgtgcacgaaccccccgttcagcccgaccgctgcgccttatccggtaactatcgtcttgagtccaacccggtaagacacgacttatcgccactggcagcagccactggtaacaggattagcagagcgaggtatgtaggcggtgctacagagttcttgaagtggtggcctaactacggctacactagaagaacagtatttggtatctgcgctctgctgaagccagttaccttcggaaaaagagttggtagctcttgatccggcaaacaaaccaccgctggtagcggtggtttttttgtttgcaagcagcagattacgcgcagaaaaaaaggatctcaagaagatcctttgatcttttctacggggtctgacgctcagtggaacgaaaactcacgttaagggattttggtcatgagattatcaaaaaggatcttcacctagatccttttaaattaaaaatgaagttttaaatcaatctaaagtatatatgagtaaacttggtctgacagttaccaatgcttaatcagtgaggcacctatctcagcgatctgtctatttcgttcatccatagttgcatttaaatttccgaactctccaaggccctcgtcggaaaatcttcaaacctttcgtccgatccatcttgcaggctacctctcgaacgaactatcgcaagtctcttggccggccttgcgccttggctattgcttggcagcgcctatcgccaggtattactccaatcccgaatatccgagatcgggatcacccgagagaagttcaacctacatcctcaatcccgatctatccgagatccgaggaatatcgaaatcggggcgcgcctggtgtaccgagaacgatcctctcagtgcgagtctcgacgatccatatcgttgcttggcagtcagccagtcggaatccagcttgggacccaggaagtccaatcgtcagatattgtactcaagcctggtcacggcagcgtaccgatctgtttaaacctagatattgatagtctgatcggtcaacgtataatcgagtcctagcttttgcaaacatctatcaagagacaggatcagcaggaggctttcgcatgagtattcaacatttccgtgtcgcccttattcccttttttgcggcattttgccttcctgtttttgctcacccagaaacgctggtgaaagtaaaagatgctgaagatcagttgggtgcgcgagtgggttacatcgaactggatctcaacagcggtaagatccttgagagttttcgccccgaagaacgctttccaatgatgagcacttttaaagttctgctatgtggcgcggtattatcccgtattgacgccgggcaagagcaactcggtcgccgcatacactattctcagaatgacttggttgagtattcaccagtcacagaaaagcatcttacggatggcatgacagtaagagaattatgcagtgctgccataaccatgagtgataacactgcggccaacttacttctgacaacgattggaggaccgaaggagctaaccgcttttttgcacaacatgggggatcatgtaactcgccttgatcgttgggaaccggagctgaatgaagccataccaaacgacgagcgtgacaccacgatgcctgtagcaatggcaacaaccttgcgtaaactattaactggcgaactacttactctagcttcccggcaacagttgatagactggatggaggcggataaagttgcaggaccacttctgcgctcggcccttccggctggctggtttattgctgataaatctggagccggtgagcgtgggtctcgcggtatcattgcagcactggggccagatggtaagccctcccgtatcgtagttatctacacgacggggagtcaggcaactatggatgaacgaaatagacagatcgctgagataggtgcctcactgattaagcattggtaaccgattctaggtgcattggcgcagaaaaaaatgcctgatgcgacgctgcgcgtcttatactcccacatatgccagattcagcaacggatacggcttccccaacttgcccacttccatacgtgtcctccttaccagaaatttatccttaagatcccgaatcgtttaaactcgactctggctctatcgaatctccgtcgtttcgagcttacgcgaacagccgtggcgctcatttgctcgtcgggcatcgaatctcgtcagctatcgtcagcttacctttttggca